European Patent Application EP 4 403 191 A1, published July 24, 2024. Title: Hetero nucleic acids comprising a 2'-modified nucleoside. Applicant: National University Corporation Tokyo Medical and Dental University. The sequence listing filed with the application follows.

SEQUENCE LISTING (65 sequences)

SEQ ID NO: 1 - DNA, 16 bp, synthetic construct
  misc_feature 1..16: note = synthetic
  misc_feature order(1..3,14..16): note = LNA
  source 1..16: mol_type = other DNA
atagtcactctggtga

SEQ ID NO: 2 - RNA, 16 nt, synthetic construct
  misc_feature 1..16: note = synthetic
  source 1..16: mol_type = other RNA
tcaccagagtgactat

SEQ ID NO: 3 - DNA, 16 bp, synthetic construct
  misc_feature 1..16: note = synthetic
  source 1..16: mol_type = other DNA
tcaccagagtgactat

SEQ ID NO: 4 - RNA, 16 nt, synthetic construct
  modified_base 1: mod_base = OTHER; note = thymine
  modified_base 10: mod_base = OTHER; note = thymine
  modified_base 14: mod_base = OTHER; note = thymine
  modified_base 16: mod_base = OTHER; note = thymine
  misc_feature order(1..3,14..16): note = 2'-O-MOE-RNA
  modified_base 2: mod_base = OTHER; note = 5-methylcytosine
  source 1..16: mol_type = other RNA
tcaccagagtgactat

SEQ ID NO: 5 - RNA, 16 nt, synthetic construct
  modified_base 1: mod_base = OTHER; note = thymine
  modified_base 10: mod_base = OTHER; note = thymine
  modified_base 14: mod_base = OTHER; note = thymine
  modified_base 16: mod_base = OTHER; note = thymine
  misc_feature 1..16: note = synthetic
  misc_feature 1..16: note = 2'-O-MOE-RNA
  misc_feature order(2,4..5,13): note = 5-methylcytosine
  source 1..16: mol_type = other RNA
tcaccagagtgactat

SEQ ID NO: 6 - DNA, 13 bp, synthetic construct
  misc_feature 1..13: note = synthetic
  misc_feature order(1..2,11..13): note = LNA
  source 1..13: mol_type = other DNA
gtattgctgagga

SEQ ID NO: 7 - RNA, 13 nt, synthetic construct
  misc_feature 1..13: note = synthetic
  source 1..13: mol_type = other RNA
tcctcagcaatac

SEQ ID NO: 8 - DNA, 13 bp, synthetic construct
  misc_feature 1..13: note = synthetic
  source 1..13: mol_type = other DNA
tcctcagcaatac

SEQ ID NO: 9 - DNA, 13 bp, synthetic construct
  misc_feature order(1..3,12..13): note = 2'-O-MOE-RNA
  modified_base order(2..3,13): mod_base = OTHER; note = 5-methylcytosine
  source 1..13: mol_type = other DNA
  misc_feature 4..11: note = DNA
  modified_base 1: mod_base = OTHER; note = thymine
tcctcagcaatac

SEQ ID NO: 10 - DNA, 20 bp, synthetic construct
  misc_feature order(1..5,16..20): note = 2'-O-MOE-RNA
  modified_base order(5,17): mod_base = OTHER; note = 5-methylcytosine
  source 1..20: mol_type = other DNA
gggtcagctgccaatgctag

SEQ ID NO: 11 - RNA, 20 nt, synthetic construct
  misc_feature 1..20: note = synthetic
  source 1..20: mol_type = other RNA
ctagcattggcagctgaccc

SEQ ID NO: 12 - DNA, 20 bp, synthetic construct
  misc_feature 1..20: note = synthetic
  source 1..20: mol_type = other DNA
ctagcattggcagctgaccc

SEQ ID NO: 13 - DNA, 20 bp, synthetic construct
  misc_feature order(1..5,16..20): note = 2'-O-MOE-RNA
  modified_base order(1,5,18..20): mod_base = OTHER; note = 5-methylcytosine
  source 1..20: mol_type = other DNA
  modified_base 2: mod_base = OTHER; note = thymine
  misc_feature 6..15: note = DNA
ctagcattggcagctgaccc

SEQ ID NO: 14 - RNA, 16 nt, synthetic construct
  modified_base 1: mod_base = OTHER; note = thymine
  modified_base 14: mod_base = OTHER; note = thymine
  modified_base 16: mod_base = OTHER; note = thymine
  misc_feature 1..16: note = synthetic
  misc_feature order(1..3,14..16): note = 2'-O-MOE-RNA
  modified_base 2: mod_base = OTHER; note = 5-methylcytosine
  source 1..16: mol_type = other RNA
tcaccagagtgactat

SEQ ID NO: 15 - DNA, 16 bp, synthetic construct
  misc_feature order(1..3,14..16): note = 2'-O-Me-RNA
  source 1..16: mol_type = other DNA
  modified_base order(1,14,16): mod_base = OTHER; note = uracil
tcaccagagtgactat

SEQ ID NO: 16 - DNA, 16 bp, synthetic construct
  misc_feature order(1..3,14..16): note = 2'F-RNA
  source 1..16: mol_type = other DNA
  modified_base order(1,14,16): mod_base = OTHER; note = uracil
tcaccagagtgactat

SEQ ID NO: 17 - DNA, 16 bp, synthetic construct
  misc_feature order(1..3,7,9,11,14..16): note = 2'-O-MOE-RNA
  modified_base 2: mod_base = OTHER; note = 5-methylcytosine
  source 1..16: mol_type = other DNA
  modified_base order(1,14,16): mod_base = OTHER; note = thymine
tcaccagagtgactat

SEQ ID NO: 18 - DNA, 16 bp, synthetic construct
  misc_feature order(1..3,14..16): note = 2'-O-MOE-RNA
  modified_base 2: mod_base = OTHER; note = 5-methylcytosine
  misc_feature order(7,9,11): note = RNA
  source 1..16: mol_type = other DNA
  modified_base order(1,14,16): mod_base = OTHER; note = thymine
tcaccagagtgactat

SEQ ID NO: 19 - DNA, 16 bp, synthetic construct
  misc_feature order(1..3,14..16): note = 2'-O-MOE-RNA
  modified_base 2: mod_base = OTHER; note = 5-methylcytosine
  modified_base order(7,9,11): mod_base = i
  source 1..16: mol_type = other DNA
  modified_base order(1,14,16): mod_base = OTHER; note = thymine
tcaccanantnactat

SEQ ID NO: 20 - DNA, 16 bp, synthetic construct
  misc_feature 1..6: note = 2'-O-MOE-RNA
  modified_base order(2,4..5): mod_base = OTHER; note = 5-methylcytosine
  source 1..16: mol_type = other DNA
  modified_base 1: mod_base = OTHER; note = thymine
tcaccagagtgactat

SEQ ID NO: 21 - DNA, 16 bp, synthetic construct
  misc_feature 11..16: note = 2'-O-MOE-RNA
  modified_base 13: mod_base = OTHER; note = 5-methylcytosine
  source 1..16: mol_type = other DNA
tcaccagagtgactat

SEQ ID NO: 22 - DNA, 16 bp, synthetic construct
  misc_feature 1..10: note = 2'-O-MOE-RNA
  modified_base order(2,4..5): mod_base = OTHER; note = 5-methylcytosine
  source 1..16: mol_type = other DNA
  modified_base order(1,10): mod_base = OTHER; note = thymine
tcaccagagtgactat

SEQ ID NO: 23 - DNA, 16 bp, synthetic construct
  misc_feature 7..16: note = 2'-O-MOE-RNA
  modified_base 13: mod_base = OTHER; note = 5-methylcytosine
  source 1..16: mol_type = other DNA
  modified_base order(10,14,16): mod_base = OTHER; note = thymine
tcaccagagtgactat

SEQ ID NO: 24 - DNA, 13 bp, synthetic construct
  misc_feature 1..5: note = 2'-O-MOE-RNA
  modified_base order(2..3,5): mod_base = OTHER; note = 5-methylcytosine
  source 1..13: mol_type = other DNA
  modified_base order(1,4): mod_base = OTHER; note = thymine
tcctcagcaatac

SEQ ID NO: 25 - DNA, 13 bp, synthetic construct
  misc_feature 9..13: note = 2'-O-MOE-RNA
  modified_base 13: mod_base = OTHER; note = 5-methylcytosine
  source 1..13: mol_type = other DNA
  modified_base 11: mod_base = OTHER; note = thymine
tcctcagcaatac

SEQ ID NO: 26 - DNA, 13 bp, synthetic construct
  misc_feature 1..8: note = 2'-O-MOE-RNA
  modified_base order(2..3,5,8): mod_base = OTHER; note = 5-methylcytosine
  source 1..13: mol_type = other DNA
  modified_base order(1,4): mod_base = OTHER; note = thymine
tcctcagcaatac

SEQ ID NO: 27 - DNA, 13 bp, synthetic construct
  misc_feature 6..13: note = 2'-O-MOE-RNA
  modified_base order(8,13): mod_base = OTHER; note = 5-methylcytosine
  source 1..13: mol_type = other DNA
  modified_base 11: mod_base = OTHER; note = thymine
tcctcagcaatac

SEQ ID NO: 28 - DNA, 13 bp, synthetic construct
  misc_feature 1..10: note = 2'-O-MOE-RNA
  modified_base order(2..3,5,8): mod_base = OTHER; note = 5-methylcytosine
  source 1..13: mol_type = other DNA
  modified_base order(1,4): mod_base = OTHER; note = 5-methylcytosine
tcctcagcaatac

SEQ ID NO: 29 - DNA, 13 bp, synthetic construct
  misc_feature 4..13: note = 2'-O-MOE-RNA
  modified_base order(5,8,13): mod_base = OTHER; note = 5-methylcytosine
  source 1..13: mol_type = other DNA
  modified_base order(4,11): mod_base = OTHER; note = thymine
tcctcagcaatac

SEQ ID NO: 30 - DNA, 16 bp, synthetic construct
  misc_feature order(1..5,13..16): note = 2'-O-MOE-RNA
  modified_base order(2,4..5,13): mod_base = OTHER; note = 5-methylcytosine
  source 1..16: mol_type = other DNA
  modified_base order(1,14,16): mod_base = OTHER; note = thymine
tcaccagagtgactat

SEQ ID NO: 31 - DNA, 16 bp, synthetic construct
  misc_feature order(1..6,12..16): note = 2'-O-MOE-RNA
  modified_base order(2,4..5,13): mod_base = OTHER; note = 5-methylcytosine
  source 1..16: mol_type = other DNA
  modified_base order(1,14,16): mod_base = OTHER; note = thymine
tcaccagagtgactat

SEQ ID NO: 32 - DNA, 16 bp, synthetic construct
  misc_feature order(1..7,11..16): note = 2'-O-MOE-RNA
  modified_base order(2,4..5,13): mod_base = OTHER; note = 5-methylcytosine
  source 1..16: mol_type = other DNA
  modified_base order(1,4,6): mod_base = OTHER; note = thymine
tcaccagagtgactat

SEQ ID NO: 33 - DNA, 16 bp, synthetic construct
  misc_feature order(1..8,10..16): note = 2'-O-MOE-RNA
  modified_base order(2,4..5,13): mod_base = OTHER; note = 5-methylcytosine
  source 1..16: mol_type = other DNA
  modified_base order(1,10,14,16): mod_base = OTHER; note = thymine
tcaccagagtgactat

SEQ ID NO: 34 - DNA, 16 bp, synthetic construct
  misc_feature order(3,6,8,12,15): note = RNA
  source 1..16: mol_type = other DNA
tcaccagagtgactat

SEQ ID NO: 35 - DNA, 16 bp, synthetic construct
  misc_feature order(7,9,11): note = RNA
  source 1..16: mol_type = other DNA
tcaccagagtgactat

SEQ ID NO: 36 - DNA, 16 bp, synthetic construct
  misc_feature order(2,4..5,13): note = RNA
  source 1..16: mol_type = other DNA
tcaccagagtgactat

SEQ ID NO: 37 - DNA, 16 bp, synthetic construct
  misc_feature order(1,10,14,16): note = RNA
  source 1..16: mol_type = other DNA
  modified_base order(1,10,14,16): mod_base = OTHER; note = uracil
tcaccagagtgactat

SEQ ID NO: 38 - DNA, 16 bp, synthetic construct
  misc_feature order(3,6..9,11..12,15): note = RNA
  source 1..16: mol_type = other DNA
tcaccagagtgactat

SEQ ID NO: 39 - DNA, 16 bp, synthetic construct
  misc_feature order(1..2,4..5,10,13..14,16): note = RNA
  source 1..16: mol_type = other DNA
  modified_base order(1,10,14,16): mod_base = OTHER; note = uracil
tcaccagagtgactat

SEQ ID NO: 40 - DNA, 20 bp, synthetic construct
  misc_feature order(3,6,12,17): note = RNA
  source 1..20: mol_type = other DNA
ctagcattggcagctgaccc

SEQ ID NO: 41 - DNA, 20 bp, synthetic construct
  misc_feature order(4,9..10,13,16): note = RNA
  source 1..20: mol_type = other DNA
ctagcattggcagctgaccc

SEQ ID NO: 42 - DNA, 20 bp, synthetic construct
  misc_feature order(1,5,11,14,18..20): note = RNA
  source 1..20: mol_type = other DNA
ctagcattggcagctgaccc

SEQ ID NO: 43 - DNA, 20 bp, synthetic construct
  misc_feature order(2,7..8,15): note = RNA
  source 1..20: mol_type = other DNA
  modified_base order(2,7..8,15): mod_base = OTHER; note = uracil
ctagcattggcagctgaccc

SEQ ID NO: 44 - DNA, 16 bp, synthetic construct
  misc_feature order(3,6,8,12,15): note = 2'-O-MOE-RNA
  source 1..16: mol_type = other DNA
tcaccagagtgactat

SEQ ID NO: 45 - DNA, 16 bp, synthetic construct
  misc_feature order(7,9,11): note = 2'-O-MOE-RNA
  source 1..16: mol_type = other DNA
tcaccagagtgactat

SEQ ID NO: 46 - DNA, 16 bp, synthetic construct
  misc_feature order(2,4..5,13): note = 2'-O-MOE-RNA
  modified_base order(2,4..5,13): mod_base = OTHER; note = 5-methylcytosine
  source 1..16: mol_type = other DNA
tcaccagagtgactat

SEQ ID NO: 47 - DNA, 16 bp, synthetic construct
  misc_feature order(1,10,14,16): note = 2'-O-MOE-RNA
  source 1..16: mol_type = other DNA
  modified_base order(1,10,14,16): mod_base = OTHER; note = thymine
tcaccagagtgactat

SEQ ID NO: 48 - DNA, 16 bp, synthetic construct
  misc_feature order(1..5,12..13): note = 2'-O-MOE-RNA
  modified_base order(2,4..5,13): mod_base = OTHER; note = 5-methylcytosine
  source 1..16: mol_type = other DNA
  modified_base 1: mod_base = OTHER; note = thymine
tcaccagagtgactat

SEQ ID NO: 49 - DNA, 16 bp, synthetic construct
  misc_feature order(2..6,13..14): note = 2'-O-MOE-RNA
  modified_base order(2,4..5,13): mod_base = OTHER; note = 5-methylcytosine
  source 1..16: mol_type = other DNA
tcaccagagtgactat

SEQ ID NO: 50 - DNA, 16 bp, synthetic construct
  misc_feature order(1..6,12..14): note = 2'-O-MOE-RNA
  modified_base order(2,4..5,13): mod_base = OTHER; note = 5-methylcytosine
  source 1..16: mol_type = other DNA
  modified_base order(1,4): mod_base = OTHER; note = thymine
tcaccagagtgactat

SEQ ID NO: 51 - DNA, 18 bp, synthetic construct
  misc_feature order(1..8,11..18): note = 2'-O-MOE-RNA
  modified_base order(2,4..5,15): mod_base = OTHER; note = 5-methylcytosine
  source 1..18: mol_type = other DNA
  modified_base order(1,14,16): mod_base = OTHER; note = thymine
tcaccagattgtgactat

SEQ ID NO: 52 - DNA, 18 bp, synthetic construct
  misc_feature order(1..7,11..18): note = 2'-O-MOE-RNA
  modified_base order(2,4..5,15): mod_base = OTHER; note = 5-methylcytosine
  source 1..18: mol_type = other DNA
  modified_base order(1,10,14,16): mod_base = OTHER; note = thymine
tcaccagtttgtgactat

SEQ ID NO: 53 - DNA, 19 bp, synthetic construct
  misc_feature order(1..8,12..19): note = 2'-O-MOE-RNA
  modified_base order(2,4..5,16): mod_base = OTHER; note = 5-methylcytosine
  source 1..19: mol_type = other DNA
  modified_base order(1,13,17,19): mod_base = OTHER; note = 5-methylcytosine
tcaccagatttgtgactat

SEQ ID NO: 54 - DNA, 35 bp, synthetic construct
  misc_feature order(1..3,14..16): note = 2'-O-MOE-RNA
  modified_base 2: mod_base = OTHER; note = 5-methylcytosine
  misc_feature order(20..22,33..35): note = LNA
  source 1..35: mol_type = other DNA
  modified_base order(1,14,16): mod_base = OTHER; note = thymine
tcaccagagtgactataaaatagtcactctggtga

SEQ ID NO: 55 - DNA, 32 bp, synthetic construct
  misc_feature order(1..3,14..16): note = 2'-O-MOE-RNA
  modified_base 2: mod_base = OTHER; note = 5-methylcytosine
  misc_feature order(17..19,30..32): note = LNA
  source 1..32: mol_type = other DNA
  modified_base order(1,14,16): mod_base = OTHER; note = thymine
tcaccagagtgactatatagtcactctggtga

SEQ ID NO: 56 - DNA, 41 bp, synthetic construct
  misc_feature order(1..5,9..14,18..22): note = 2'-O-MOE-RNA
  modified_base order(2,4..5,19): mod_base = OTHER; note = 5-methylcytosine
  misc_feature order(26..28,39..41): note = LNA
  source 1..41: mol_type = other DNA
  modified_base order(1,13,20,22): mod_base = OTHER; note = thymine
tcacctttagagtgtttactataaaatagtcactctggtga

SEQ ID NO: 57 - RNA, 20 nt, synthetic construct
  source 1..20: mol_type = other RNA
  misc_feature order(1..5,16..20): note = 2'-O-MOE-RNA
  modified_base order(1,5,18..20): mod_base = OTHER; note = 5-methylcytosine
ctagcattggcagctgaccc

SEQ ID NO: 58 - DNA, 20 bp, synthetic construct
  misc_feature order(1..5,16..20): note = 2'-O-MOE-RNA
  source 1..20: mol_type = other DNA
  modified_base order(1,5,18..20): mod_base = OTHER; note = 5-methylcytosine
  misc_feature order(6,9,10,12..13): note = RNA
ctagcattggcagctgaccc

SEQ ID NO: 59 - RNA, 20 nt, synthetic construct
  source 1..20: mol_type = other RNA
  misc_feature 6..15: note = 2'-O-MOE-RNA
  modified_base order(7..8,15): mod_base = OTHER; note = thymine
  modified_base order(11,14): mod_base = OTHER; note = 5-methylcytosine
ctagcattggcagctgaccc

SEQ ID NO: 60 - DNA, 20 bp, synthetic construct
  source 1..20: mol_type = other DNA
  misc_feature 6..15: note = 2'-O-MOE-RNA
  modified_base order(7..8,15): mod_base = OTHER; note = 5-methylcytosine
  modified_base 11..14: mod_base = OTHER; note = 5-methylcytosine
ctagcattggcagctgaccc

SEQ ID NO: 61 - DNA, 16 bp, synthetic construct
  misc_feature order(6..9,11..12): note = RNA
  source 1..16: mol_type = other DNA
  misc_feature order(1..3,14..16): note = 2'-O-MOE-RNA
  modified_base order(1,14,16): mod_base = OTHER; note = thymine
  modified_base 2: mod_base = OTHER; note = 5-methylcytosine
tcaccagagtgactat

SEQ ID NO: 62 - RNA, 18 nt, synthetic construct
  source 1..18: mol_type = other RNA
  misc_feature 1..18: note = 2'-O-MOE-RNA
  modified_base order(2,5,11): mod_base = OTHER; note = 5-methylcytosine
  modified_base order(1,3,16,18): mod_base = OTHER; note = thymine
tctacagaagcaaggtgt

SEQ ID NO: 63 - DNA, 18 bp, synthetic construct
  source 1..18: mol_type = other DNA
acaccttgcttctgtaga

SEQ ID NO: 64 - DNA, 18 bp, synthetic construct
  source 1..18: mol_type = other DNA
  misc_feature order(1..3,16..18): note = 2'-O-MOE-RNA
  modified_base 2: mod_base = OTHER; note = 5-methylcytosine
  misc_feature order(8,14): note = RNA
acaccttgcttctgtaga

SEQ ID NO: 65 - DNA, 36 bp, synthetic construct
  misc_feature order(24..25,34..36): note = LNA
  source 1..36: mol_type = other DNA
  misc_feature order(1..3,7..13,17..19): note = 2'-O-MOE-RNA
  modified_base order(2..3,8,11,19): mod_base = OTHER; note = 5-methylcytosine
  modified_base order(1,7,17): mod_base = OTHER; note = thymine
tccaaatcagcaaccctacaaaagtattgctgagga